European Patent Specification EP 3 475 420 B1, published July 16, 2025. Title: Protease Formulation. Applicant: ew Nutrition. The sequence listing filed with the application follows.

SEQUENCE LISTING (4 sequences)

SEQ ID NO: 1 - DNA, 1659 bp, Artificial
  Kumamolisin AS codon optimited for Bacillus subtilis
tcagatatggaaaaaccgtggaaagaaggcgaagaagctagagcagttctgcaaggccatgcaagagcacaagcaccgcaagcagttgataaaggaccggttgcaggcgacgaaagaatggcagttacagttgttctgcgcagacaaagagcaggcgaactggcagcacatgttgaaagacaagcagcaattgcaccgcatgcaagagaacatctgaaaagagaagcatttgcagcatcacatggcgcatcactggatgattttgcagaactgagaagatttgcagatgcgcatggcctggcactggatagagcaaatgttgcagcaggcacagcagttctgtcaggaccggttgatgcaattaatagagcatttggcgttgaactgcgccattttgatcatccggatggctcatatagatcatatctgggcgaagttacagttccggcatcaattgcaccgatgattgaagcagttctgggcctggatacaagaccggttgcaagaccgcattttagaatgcaaagacgcgcagaaggcggatttgaagcaagatcacaagcagcagcaccgacagcatatacaccgctggatgttgcacaagcatatcaatttccggaaggcctggatggacaaggccaatgcattgcaattattgaacttggcggaggctatgatgaagcatcactggcacaatattttgcatcactgggcgttccggcaccgcaagttgtttcagtttcagttgatggcgcatcaaatcaaccgacaggcgatccgtcaggaccggatggcgaagttgaactggatattgaagttgcaggcgcactggcacctggcgcaaaatttgcagtttattttgcaccgaatacggatgcaggctttctggatgcaattacaacagcaattcatgatccgacactgaaaccgtcagttgtttcaattagctggggaggaccggaagattcatggacatcagcagcgattgcagcaatgaatagagcgtttcttgatgcagcagcactgggcgttacagttctggcagcagcaggcgattcaggcagcacagatggcgaacaagatggcctgtatcatgttgattttccggcagcatcaccgtatgttctggcatgcggaggcacaagacttgttgcatcaggcggaagaattgcacaagaaacagtttggaatgatggacctgatggcggagcaacaggcggaggcgtttcaagaatttttccgcttccggcatggcaagaacatgcaaatgttccgccttcagcaaatcctggcgcatcatcaggcagaggcgttccggatctggcaggcaatgcagatccggcaacaggctatgaagttgttattgatggcgaagcgacagttattggcggaacatcagcagttgcaccgctgtttgcagcactggttgcaagaattaatcaaaaactgggcaaagcagtcggctatctgaatccgacactgtatcaacttccggcagatgtctttcatgatattacagaaggcaacaacgatattgcgaatcgcgcacaaatttatcaagcaggaccgggatgggatccgtgcacaggcctgggctcaccgattggcgttagactgctgcaagcactgctgccgtcagcatcacaaccgcaaccgtaa

SEQ ID NO: 2 - DNA, 795 bp, Artificial
  Aspergillopepsin 2 codon optimized for S.cerevisiae
gctccattgactgaaaaaagaagagctagaaaagaagctagagctgctggtaagagacattctaatccaccatatattccaggttccgacaaagaaatcttgaagttgaacggtactaccaacgaagaatactcttctaattgggctggtgctgttttgattggtgatggttatacaaaggttaccggtgaattcactgttccatctgtttctgctggttcttcaggttcttctggttatggtggtggttacggttattggaaaaacaagagacaatccgaagaatattgtgcttctgcttgggttggtattgatggtgatacttgtgaaactgctatcttgcaaactggtgttgatttctgttacgaagatggtcaaacttcttacgatgcttggtatgaatggtatccagattacgcttacgatttctccgatattaccatctctgaaggtgattccatcaaggttactgttgaagctacctctaaatcatctggttctgccactgttgaaaacttgactactggtcaatctgttacccatactttctctggtaatgttgaaggtgacttgtgtgaaactaatgccgaatggatcgttgaagatttcgaatctggtgattctttggttgcttttgctgatttcggttctgttactttcactaacgctgaagctacttctggtggttctactgttggtccatctgatgctactgttatggatattgaacaagacggttccgttttgaccgaaacttctgtttcaggtgattctgttaccgttacttacgtttga

SEQ ID NO: 3 - DNA, 1746 bp, artificial
  Grifolisin codon optimized for Saccharomyces cerevisiae
actccaagagttccattgtccgaacaatctcatccttccaatatgatcacctcttctttcttggttgtctccttgtttactttggctttgtctaagccaatgtccagatctatgaaggttcacgaaactagagaaggtattccagatggttttgctttggctggttctccttcttctgatacttctttgaacttgagaattgccttggtccaaaatgatccagctggtttggaaactgcattatacgatgttaataccccatcctctgctaactacggtaaccatttgtctaaagccgaagttgaaaagttcgttgctccagaaccagaatctgttgatgctgttaatgcttggttggaagaaaatggtttgactgctactactatttctcctgctggtgattggttggcttttgaagttccagtttctaaggccaacgaattattcgatgctgatttctctgtttacacccatactgatactggtttagaagccattagaaccttgtcctattctattccagctgaattgcaaggtcacttggatttggttcatccaactattactttcccaaacccatactcaagattgccagttgttgcttcttctattaagactgctgctccaacttctgataacttgacttctttggctgttccatcttcttgtgcttctacaattactccagcttgtttacaagccttgtacggtattccaactacaccagctactcaatcttctaacaaattggctgtttccggttacattgaacaattcgctaatcaagccgacttgaaaactttcttgactaagttcagaaccgacatctcttcttctactactttcactactcaaaccttggatggtggtgaaaatccacaaaatggtaatgaagctggtgttgaagctgatttggatgttcaatatactgttggtttggctactgatgttccaaccgttttcatttctgttggtgataactttcaagacggtgctttggaaggtttcttggacattatcaatttcttgttggacgaatctaccccacctcaagttttgactacttcttatggtcaaaacgaaaacaccatctccagaaacttggctaacaatttgtgtaacgcttacgctcaattgggtgctagaggtacttctattttgtttgcttcaggtgacggtggtgtttctggttcacaatctgattcttgttctaagttcgttccaactttcccatctggttgtccttttatgacttcagttggtgctactacaggtattaacccagaaactgctgctgatttttcttctggtggtttctctaattacttcggtactccatcttatcaagcctctgctcattctgcttacttgcaagccttgggttctactaatgctggtaagtttaatacctctggtagaggttttccagacgtttctactcaaggtgaaaacttccaaatcgttgttgatggtcaaaccggtacagttgatggtacatcatgtgcttctccaacctttgcttctgttgtttctttgttgaacgatagattgattgctgccggtaaatctccattgggttttttgaatccattcttgtactctactggtgcttctgcctttaactctattacatctggttctaacccaggttgtaacactaatggtttcccagctaaaactggttggtcaccagttactggtttgggtactccaaattttgctaagttgttaaccgccgttggttta

SEQ ID NO: 4 - DNA, 795 bp, artificial; identical to SEQ ID NO: 2
  Aspergillopepsin 2 codon optimized for Hansenula polymorpha